European Patent Specification EP 3 085 786 B1, published July 23, 2025. Title: Use of aptamers in therapy and/or diagnosis of autoimmunediseases. Applicant: Charite - Universitätsmedizin Berlin Max-Delbrück-Centrum für Molekulare Medizin. The sequence listing filed with the application follows.

SEQUENCE LISTING (3 sequences)

SEQ ID NO: 1 - DNA, 15 bp, artificial
  aptamer sequence 1
ggttggtgtggttgg

SEQ ID NO: 2 - DNA, 26 bp, artificial
  aptamer sequence 2
cgcctaggttgggtagggtggtggcg

SEQ ID NO: 3 - DNA, 12 bp, artificial
  truncated 12mer of SEQ ID No. 1
ggttggtgtggt